European Patent Specification EP 3 274 362 B1, published August 27, 2025. Title: NOUVEAU PROCEDE PERMETTANT DE FAVORISER LA NODULATION CHEZ LES PLANTES. Applicant: UNIVERSITE TOULOUSE III - PAUL SABATIER CENTRE NATIONAL DE LA RECHERCHE SCIENTIFIQUE - CNRS. The sequence listing filed with the application follows.

SEQUENCE LISTING (9 sequences)

SEQ ID NO: 1 - RNA, 21 nt, Glycine max
ggaaucuugaugaugcugcag

SEQ ID NO: 2 - protein, 16 aa, Glycine max
MWVLCLFCWPTYTHGS

SEQ ID NO: 3 - DNA, 51 bp, Glycine max
atgtgggtcttgtgtttgttttgttggcctacatatacacatgggagttga

SEQ ID NO: 4 - DNA, 929 bp, Glycine max
cactctctcatctctacttgaccactctctctatatatacaccactaaaccctttcttcgttctcagttatcttctttcacttcacttaacctagcctccttcccattctgatttgagttcttgctttgcctcttaattttatttttcctcttagctttcttcgatcttaacctttgaacagtaattgcttgctttgtatacattaattactataggtggtactttggcagcttttctattgtatagagacttatcagtgaataatactactatgtgggtcttgtgtttgttttgttggcctacatatacacatgggagttgaggagccttttaggccttagccttacattagttgtccctctttccttgcctttacttttgcttcatatattggatttgattagatttagggttagggttagggctgttctattctcctcctcctccttttctacttcctgatatgcttcaattcctcctctctctctctctctcttgaagttttatgttttatggccaagtgatcttaatggtggtaacacagagagacctaatgaagtcctaaataaactaaagaaatcagtcactgtttgccggtggagcatcatcaagattcacaagctttaggggcattaatttgtttgaggtggttccttattgctccaaaaccaattagcccttttgctatgggaatcttgatgatgctgcagcagcaataaatgactaatactactaccagatattgcttgaggaggatctcactactacacaactgtgctacaaggccaggagcaaaggaggttatttaattaactaaataattatgttattaatttgttttctaaatattcaagaaattggattaggtaattaccaagttacaagccacttttggatttacctttattaactctagtagctgataaat

SEQ ID NO: 5 - protein, 16 aa, Artificial sequence
  Synthetic peptide
VLWCSHCMGFLWPTYT

SEQ ID NO: 6 - RNA, 21 nt, Glycine max
ugaagcugccagcaugaucug

SEQ ID NO: 7 - protein, 17 aa, Glycine max
MKGVHHFFHHKYVGLRG

SEQ ID NO: 8 - DNA, 51 bp, Glycine max
atgaaaggggttcatcacttttttcatcacaagtatgttggtttgagaggt

SEQ ID NO: 9 - DNA, 665 bp, Glycine max
gaaaaggaagtcattgtcaatagctgtaaggaggagcaaaacctaccattaaatactccctctatggcacagtagtgaaagaaaagagacattgagctgcgcacaggcattcattcatatggatcagtgtggagataaagaggatcacgagggtctccctttaattactccaaacatgcatggcttgttcccctttttgttaatttctatgtatcaagatgttggtaccctctctcaggatttgcttcaatgaaaggggttcatcacttttttcatcacaagtatgttggtttgagaggttgaagctgccagcatgatctggtaaatcacatacttttttttttctcacctctcatgcctaatttttaagcaccagtcattagagaaaataatggtgaaaaatccatctattcaattttttttttcaaattcaaggtttccagtatgtatcactaatggtgaaaaaagtgatggaattttgtagaacatgggttaaatttactttttttttttttgagttttcattttcttcaagtttctgagccaagaaataaaagagacttataaattggaattaatacttaaaggaaacccaccagaagggcaatttggttatcataagatgtggtttccatcaggtcatcttgcagcttcaatcactcaat